European Patent Specification EP 3 464 347 B1, published May 31, 2023. Title: CYSTEINE OPTIMIZED IMPROVEMENTS TO MULTIMERIZING STRADOMERS. Applicant: Block, David S. Olsen, Henrik. The sequence listing filed with the application follows.

SEQUENCE LISTING (44 sequences)

SEQ ID NO: 1 - protein, 20 aa, Artificial Sequence
  leader sequence
METDTLLLWVLLLWVPGSTG

SEQ ID NO: 2 - protein, 232 aa, Homo sapiens
EPKSCDKTHTCPPCPAPELLGGPSVFLFPPKPKDTLMISRTPEVTCVVVDVSHEDPEVKFNWYVDGVEVHNAKTKPREEQYNSTYRVVSVLTVLHQDWLNGKEYKCKVSNKALPAPIEKTISKAKGQPREPQVYTLPPSREEMTKNQVSLTCLVKGFYPSDIAVEWESNGQPENNYKTTPPVLDSDGSFFLYSKLTVDKSRWQQGNVFSCSVMHEALHNHYTQKSLSLSPGK

SEQ ID NO: 3 - protein, 40 aa, Homo sapiens
GGGSIKQIEDKIEEILSKIYHIENEIARIKKLIGERGHDI

SEQ ID NO: 4 - protein, 38 aa, Homo sapiens
GGGSIKQIEDKIEEILSKIYHIENEIARIKKLIGERGH

SEQ ID NO: 5 - protein, 34 aa, Homo sapiens
IKQIEDKIEEILSKIYHIENEIARIKKLIGERGH

SEQ ID NO: 6 - protein, 36 aa, Homo sapiens
GGGSIKQIEDKIEEILSKIYHIENEIARIKKLIGER

SEQ ID NO: 7 - protein, 32 aa, Homo sapiens
IKQIEDKIEEILSKIYHIENEIARIKKLIGER

SEQ ID NO: 8 - protein, 12 aa, Homo sapiens
ERKCCVECPPCP

SEQ ID NO: 9 - protein, 15 aa, Homo sapiens
EPKSCDKTHTCPPCP

SEQ ID NO: 10 - protein, 244 aa, Homo sapiens
EPKSCDKTHTCPPCPAPELLGGPSVFLFPPKPKDTLMISRTPEVTCVVVDVSHEDPEVKFNWYVDGVEVHNAKTKPREEQYNSTYRVVSVLTVLHQDWLNGKEYKCKVSNKALPAPIEKTISKAKGQPREPQVYTLPPSREEMTKNQVSLTCLVKGFYPSDIAVEWESNGQPENNYKTTPPVLDSDGSFFLYSKLTVDKSRWQQGNVFSCSVMHEALHNHYTQKSLSLSPGKERKCCVECPPCP

SEQ ID NO: 11 - protein, 15 aa, Homo sapiens
EPKSSDKTHTCPPCP

SEQ ID NO: 12 - protein, 15 aa, Homo sapiens
EPKSCDKTHTSPPCP

SEQ ID NO: 13 - protein, 15 aa, Homo sapiens
EPKSCDKTHTCPPSP

SEQ ID NO: 14 - protein, 217 aa, Homo sapiens
APELLGGPSVFLFPPKPKDTLMISRTPEVTSVVVDVSHEDPEVKFNWYVDGVEVHNAKTKPREEQYNSTYRVVSVLTVLHQDWLNGKEYKCKVSNKALPAPIEKTISKAKGQPREPQVYTLPPSREEMTKNQVSLTCLVKGFYPSDIAVEWESNGQPENNYKTTPPVLDSDGSFFLYSKLTVDKSRWQQGNVFSCSVMHEALHNHYTQKSLSLSPGK

SEQ ID NO: 15 - protein, 217 aa, Homo sapiens
APELLGGPSVFLFPPKPKDTLMISRTPEVTCVVVDVSHEDPEVKFNWYVDGVEVHNAKTKPREEQYNSTYRVVSVLTVLHQDWLNGKEYKSKVSNKALPAPIEKTISKAKGQPREPQVYTLPPSREEMTKNQVSLTCLVKGFYPSDIAVEWESNGQPENNYKTTPPVLDSDGSFFLYSKLTVDKSRWQQGNVFSCSVMHEALHNHYTQKSLSLSPGK

SEQ ID NO: 16 - protein, 217 aa, Homo sapiens
APELLGGPSVFLFPPKPKDTLMISRTPEVTCVVVDVSHEDPEVKFNWYVDGVEVHNAKTKPREEQYNSTYRVVSVLTVLHQDWLNGKEYKCKVSNKALPAPIEKTISKAKGQPREPQVYTLPPSREEMTKNQVSLTSLVKGFYPSDIAVEWESNGQPENNYKTTPPVLDSDGSFFLYSKLTVDKSRWQQGNVFSCSVMHEALHNHYTQKSLSLSPGK

SEQ ID NO: 17 - protein, 217 aa, Homo sapiens
APELLGGPSVFLFPPKPKDTLMISRTPEVTCVVVDVSHEDPEVKFNWYVDGVEVHNAKTKPREEQYNSTYRVVSVLTVLHQDWLNGKEYKCKVSNKALPAPIEKTISKAKGQPREPQVYTLPPSREEMTKNQVSLTCLVKGFYPSDIAVEWESNGQPENNYKTTPPVLDSDGSFFLYSKLTVDKSRWQQGNVFSSSVMHEALHNHYTQKSLSLSPGK

SEQ ID NO: 18 - protein, 12 aa, Homo sapiens
ERKCCVESPPCP

SEQ ID NO: 19 - protein, 12 aa, Homo sapiens
ERKCSVECPPCP

SEQ ID NO: 20 - protein, 12 aa, Homo sapiens
ERKSCVECPPCP

SEQ ID NO: 21 - protein, 12 aa, Homo sapiens
ERKCCVECPPSP

SEQ ID NO: 22 - protein, 15 aa, Homo sapiens
EPKSCDKTHTSPPSP

SEQ ID NO: 23 - protein, 15 aa, Homo sapiens
EPKSSDKTHTCPPSP

SEQ ID NO: 24 - protein, 15 aa, Homo sapiens
EPKSSDKTHTSPPCP

SEQ ID NO: 25 - protein, 15 aa, Homo sapiens
EPKSSDKTHTSPPSP

SEQ ID NO: 26 - protein, 217 aa, Homo sapiens
APELLGGPSVFLFPPKPKDTLMISRTPEVTCVVVDVSHEDPEVKFNWYVDGVEVHNAKTKPREEQYNSTYRVVSVLTVLHQDWLNGKEYKCKVSNKALPAPIEKTISKAKGQPREPQVYTLPPSREEMTKNQVSLTSLVKGFYPSDIAVEWESNGQPENNYKTTPPVLDSDGSFFLYSKLTVDKSRWQQGNVFSSSVMHEALHNHYTQKSLSLSPGK

SEQ ID NO: 27 - protein, 264 aa, Homo sapiens
METDTLLLWVLLLWVPGSTGEPKSSDKTHTCPPCPAPELLGGPSVFLFPPKPKDTLMISRTPEVTCVVVDVSHEDPEVKFNWYVDGVEVHNAKTKPREEQYNSTYRVVSVLTVLHQDWLNGKEYKCKVSNKALPAPIEKTISKAKGQPREPQVYTLPPSREEMTKNQVSLTCLVKGFYPSDIAVEWESNGQPENNYKTTPPVLDSDGSFFLYSKLTVDKSRWQQGNVFSCSVMHEALHNHYTQKSLSLSPGKERKCCVECPPCP

SEQ ID NO: 28 - protein, 264 aa, Homo sapiens
METDTLLLWVLLLWVPGSTGEPKSCDKTHTSPPCPAPELLGGPSVFLFPPKPKDTLMISRTPEVTCVVVDVSHEDPEVKFNWYVDGVEVHNAKTKPREEQYNSTYRVVSVLTVLHQDWLNGKEYKCKVSNKALPAPIEKTISKAKGQPREPQVYTLPPSREEMTKNQVSLTCLVKGFYPSDIAVEWESNGQPENNYKTTPPVLDSDGSFFLYSKLTVDKSRWQQGNVFSCSVMHEALHNHYTQKSLSLSPGKERKCCVECPPCP

SEQ ID NO: 29 - protein, 264 aa, Homo sapiens
METDTLLLWVLLLWVPGSTGEPKSCDKTHTCPPSPAPELLGGPSVFLFPPKPKDTLMISRTPEVTCVVVDVSHEDPEVKFNWYVDGVEVHNAKTKPREEQYNSTYRVVSVLTVLHQDWLNGKEYKCKVSNKALPAPIEKTISKAKGQPREPQVYTLPPSREEMTKNQVSLTCLVKGFYPSDIAVEWESNGQPENNYKTTPPVLDSDGSFFLYSKLTVDKSRWQQGNVFSCSVMHEALHNHYTQKSLSLSPGKERKCCVECPPCP

SEQ ID NO: 30 - protein, 264 aa, Homo sapiens
METDTLLLWVLLLWVPGSTGEPKSCDKTHTCPPCPAPELLGGPSVFLFPPKPKDTLMISRTPEVTCVVVDVSHEDPEVKFNWYVDGVEVHNAKTKPREEQYNSTYRVVSVLTVLHQDWLNGKEYKCKVSNKALPAPIEKTISKAKGQPREPQVYTLPPSREEMTKNQVSLTCLVKGFYPSDIAVEWESNGQPENNYKTTPPVLDSDGSFFLYSKLTVDKSRWQQGNVFSCSVMHEALHNHYTQKSLSLSPGKERKCCVESPPCP

SEQ ID NO: 31 - protein, 264 aa, Homo sapiens
METDTLLLWVLLLWVPGSTGEPKSCDKTHTCPPCPAPELLGGPSVFLFPPKPKDTLMISRTPEVTCVVVDVSHEDPEVKFNWYVDGVEVHNAKTKPREEQYNSTYRVVSVLTVLHQDWLNGKEYKCKVSNKALPAPIEKTISKAKGQPREPQVYTLPPSREEMTKNQVSLTCLVKGFYPSDIAVEWESNGQPENNYKTTPPVLDSDGSFFLYSKLTVDKSRWQQGNVFSCSVMHEALHNHYTQKSLSLSPGKERKCSVECPPCP

SEQ ID NO: 32 - protein, 264 aa, Homo sapiens
METDTLLLWVLLLWVPGSTGEPKSCDKTHTCPPCPAPELLGGPSVFLFPPKPKDTLMISRTPEVTCVVVDVSHEDPEVKFNWYVDGVEVHNAKTKPREEQYNSTYRVVSVLTVLHQDWLNGKEYKCKVSNKALPAPIEKTISKAKGQPREPQVYTLPPSREEMTKNQVSLTCLVKGFYPSDIAVEWESNGQPENNYKTTPPVLDSDGSFFLYSKLTVDKSRWQQGNVFSCSVMHEALHNHYTQKSLSLSPGKERKSCVECPPCP

SEQ ID NO: 33 - protein, 264 aa, Homo sapiens
METDTLLLWVLLLWVPGSTGEPKSCDKTHTCPPCPAPELLGGPSVFLFPPKPKDTLMISRTPEVTCVVVDVSHEDPEVKFNWYVDGVEVHNAKTKPREEQYNSTYRVVSVLTVLHQDWLNGKEYKCKVSNKALPAPIEKTISKAKGQPREPQVYTLPPSREEMTKNQVSLTCLVKGFYPSDIAVEWESNGQPENNYKTTPPVLDSDGSFFLYSKLTVDKSRWQQGNVFSCSVMHEALHNHYTQKSLSLSPGKERKCCVECPPSP

SEQ ID NO: 34 - protein, 264 aa, Homo sapiens
METDTLLLWVLLLWVPGSTGEPKSCDKTHTSPPSPAPELLGGPSVFLFPPKPKDTLMISRTPEVTCVVVDVSHEDPEVKFNWYVDGVEVHNAKTKPREEQYNSTYRVVSVLTVLHQDWLNGKEYKCKVSNKALPAPIEKTISKAKGQPREPQVYTLPPSREEMTKNQVSLTCLVKGFYPSDIAVEWESNGQPENNYKTTPPVLDSDGSFFLYSKLTVDKSRWQQGNVFSCSVMHEALHNHYTQKSLSLSPGKERKCCVECPPCP

SEQ ID NO: 35 - protein, 264 aa, Homo sapiens
METDTLLLWVLLLWVPGSTGEPKSSDKTHTCPPSPAPELLGGPSVFLFPPKPKDTLMISRTPEVTCVVVDVSHEDPEVKFNWYVDGVEVHNAKTKPREEQYNSTYRVVSVLTVLHQDWLNGKEYKCKVSNKALPAPIEKTISKAKGQPREPQVYTLPPSREEMTKNQVSLTCLVKGFYPSDIAVEWESNGQPENNYKTTPPVLDSDGSFFLYSKLTVDKSRWQQGNVFSCSVMHEALHNHYTQKSLSLSPGKERKCCVECPPCP

SEQ ID NO: 36 - protein, 264 aa, Homo sapiens
METDTLLLWVLLLWVPGSTGEPKSSDKTHTSPPCPAPELLGGPSVFLFPPKPKDTLMISRTPEVTCVVVDVSHEDPEVKFNWYVDGVEVHNAKTKPREEQYNSTYRVVSVLTVLHQDWLNGKEYKCKVSNKALPAPIEKTISKAKGQPREPQVYTLPPSREEMTKNQVSLTCLVKGFYPSDIAVEWESNGQPENNYKTTPPVLDSDGSFFLYSKLTVDKSRWQQGNVFSCSVMHEALHNHYTQKSLSLSPGKERKCCVECPPCP

SEQ ID NO: 37 - protein, 264 aa, Homo sapiens
METDTLLLWVLLLWVPGSTGEPKSSDKTHTSPPSPAPELLGGPSVFLFPPKPKDTLMISRTPEVTCVVVDVSHEDPEVKFNWYVDGVEVHNAKTKPREEQYNSTYRVVSVLTVLHQDWLNGKEYKCKVSNKALPAPIEKTISKAKGQPREPQVYTLPPSREEMTKNQVSLTCLVKGFYPSDIAVEWESNGQPENNYKTTPPVLDSDGSFFLYSKLTVDKSRWQQGNVFSCSVMHEALHNHYTQKSLSLSPGKERKCCVECPPCP

SEQ ID NO: 38 - protein, 264 aa, Homo sapiens
METDTLLLWVLLLWVPGSTGEPKSCDKTHTCPPCPAPELLGGPSVFLFPPKPKDTLMISRTPEVTSVVVDVSHEDPEVKFNWYVDGVEVHNAKTKPREEQYNSTYRVVSVLTVLHQDWLNGKEYKCKVSNKALPAPIEKTISKAKGQPREPQVYTLPPSREEMTKNQVSLTCLVKGFYPSDIAVEWESNGQPENNYKTTPPVLDSDGSFFLYSKLTVDKSRWQQGNVFSCSVMHEALHNHYTQKSLSLSPGKERKCCVECPPCP

SEQ ID NO: 39 - protein, 264 aa, Homo sapiens
METDTLLLWVLLLWVPGSTGEPKSCDKTHTCPPCPAPELLGGPSVFLFPPKPKDTLMISRTPEVTCVVVDVSHEDPEVKFNWYVDGVEVHNAKTKPREEQYNSTYRVVSVLTVLHQDWLNGKEYKSKVSNKALPAPIEKTISKAKGQPREPQVYTLPPSREEMTKNQVSLTCLVKGFYPSDIAVEWESNGQPENNYKTTPPVLDSDGSFFLYSKLTVDKSRWQQGNVFSCSVMHEALHNHYTQKSLSLSPGKERKCCVECPPCP

SEQ ID NO: 40 - protein, 264 aa, Homo sapiens
METDTLLLWVLLLWVPGSTGEPKSCDKTHTCPPCPAPELLGGPSVFLFPPKPKDTLMISRTPEVTCVVVDVSHEDPEVKFNWYVDGVEVHNAKTKPREEQYNSTYRVVSVLTVLHQDWLNGKEYKCKVSNKALPAPIEKTISKAKGQPREPQVYTLPPSREEMTKNQVSLTSLVKGFYPSDIAVEWESNGQPENNYKTTPPVLDSDGSFFLYSKLTVDKSRWQQGNVFSCSVMHEALHNHYTQKSLSLSPGKERKCCVECPPCP

SEQ ID NO: 41 - protein, 264 aa, Homo sapiens
METDTLLLWVLLLWVPGSTGEPKSCDKTHTCPPCPAPELLGGPSVFLFPPKPKDTLMISRTPEVTCVVVDVSHEDPEVKFNWYVDGVEVHNAKTKPREEQYNSTYRVVSVLTVLHQDWLNGKEYKCKVSNKALPAPIEKTISKAKGQPREPQVYTLPPSREEMTKNQVSLTCLVKGFYPSDIAVEWESNGQPENNYKTTPPVLDSDGSFFLYSKLTVDKSRWQQGNVFSSSVMHEALHNHYTQKSLSLSPGKERKCCVECPPCP

SEQ ID NO: 42 - protein, 264 aa, Homo sapiens
METDTLLLWVLLLWVPGSTGEPKSCDKTHTCPPCPAPELLGGPSVFLFPPKPKDTLMISRTPEVTCVVVDVSHEDPEVKFNWYVDGVEVHNAKTKPREEQYNSTYRVVSVLTVLHQDWLNGKEYKCKVSNKALPAPIEKTISKAKGQPREPQVYTLPPSREEMTKNQVSLTSLVKGFYPSDIAVEWESNGQPENNYKTTPPVLDSDGSFFLYSKLTVDKSRWQQGNVFSSSVMHEALHNHYTQKSLSLSPGKERKCCVECPPCP

SEQ ID NO: 43 - protein, 9 aa, Homo sapiens
CCVECPPCP

SEQ ID NO: 44 - protein, 12 aa, Homo sapiens
SCDKTHTCPPCP